European Patent Specification EP 3 704 219 B1, published January 10, 2024. Title: Polypeptides and compositions comprising such polypeptides. Applicant: Novozymes A/S. The sequence listing filed with the application follows.

SEQUENCE LISTING (18 sequences)

SEQ ID NO: 1 - DNA, 1086 bp, Lactobacillus paraplantarum
  CDS (1)..(1083)
  sig_peptide (1)..(90)
  mat_peptide (91)..(1083)
atgaagtaccgacattactttacacaactattaatatttattagcccgctgattcttctttgcttcagccagccccgtacggcaactgccaattcatcaacattgaatactagtcaaggggtcatgttagatttaggccgccatccgttagatgaaactgcaattaaagccgtcattagtgctgctgccgaacaacacatgcaatacgtcgaactacacttatcagataacgaacatctatgctttcaatcggcttatttaggtaatgccgcatcggcaaccgtattatcggcgacgactttagaacagctagttgcttatgccaatcagttgaacattgaactagttcctgatgttgaccttccctcgcacgcgggagccattttacgccaattgcaacaaactcatcccgatatttacaataccgttaagttggatgacgaaaccatcgactatactaaaccggcagcaatcagtctcgctaccacactttatggcgagctcgatgctagttttaacaatcaaagccagcacgatttgatgctcggcgctgatgaggttcctggcagcgctagcgcctatatcgaactgaccacctttatcaatcaggtcagtcgatttcaaaatcaacacggcttcaacactagtatttggaatgattcgctattaaaaaatgaactcactcgtctggattcaaacattacaatcaattactggtcacaatctggtaacaataccgatgtggctatcattgccgaccgctatgccaaccgtgtatccgttcccgacattttagcctctgggcatccgatcgtgaactgtaatagttatgcgacctattatcaaatcaaaaatattggcaatgtcaatgatgacgattactttattaattatcttaatcacacctttcgcccgaatatctttaacgaaattgacaccaatgggcataatcaggattggaccattgaagatggcgtcacaactaacggtatcttagttagcttgtggggggccgattcagagcatgttacaccaactgccatcgtcaatttcattaaacgtatgacgattccacggtcattttaa

SEQ ID NO: 2 - protein, 361 aa, Lactobacillus paraplantarum
MKYRHYFTQLLIFISPLILLCFSQPRTATANSSTLNTSQGVMLDLGRHPLDETAIKAVISAAAEQHMQYVELHLSDNEHLCFQSAYLGNAASATVLSATTLEQLVAYANQLNIELVPDVDLPSHAGAILRQLQQTHPDIYNTVKLDDETIDYTKPAAISLATTLYGELDASFNNQSQHDLMLGADEVPGSASAYIELTTFINQVSRFQNQHGFNTSIWNDSLLKNELTRLDSNITINYWSQSGNNTDVAIIADRYANRVSVPDILASGHPIVNCNSYATYYQIKNIGNVNDDDYFINYLNHTFRPNIFNEIDTNGHNQDWTIEDGVTTNGILVSLWGADSEHVTPTAIVNFIKRMTIPRSF

SEQ ID NO: 3 - protein, 331 aa, Lactobacillus paraplantarum
NSSTLNTSQGVMLDLGRHPLDETAIKAVISAAAEQHMQYVELHLSDNEHLCFQSAYLGNAASATVLSATTLEQLVAYANQLNIELVPDVDLPSHAGAILRQLQQTHPDIYNTVKLDDETIDYTKPAAISLATTLYGELDASFNNQSQHDLMLGADEVPGSASAYIELTTFINQVSRFQNQHGFNTSIWNDSLLKNELTRLDSNITINYWSQSGNNTDVAIIADRYANRVSVPDILASGHPIVNCNSYATYYQIKNIGNVNDDDYFINYLNHTFRPNIFNEIDTNGHNQDWTIEDGVTTNGILVSLWGADSEHVTPTAIVNFIKRMTIPRSF

SEQ ID NO: 4 - DNA, 1146 bp, Lactobacillus apinorum
  CDS (1)..(1143)
  sig_peptide (1)..(84)
  mat_peptide (85)..(1143)
atgagaaataaacgatttataatcgttggaatgatattgtttttagtcttaatgtttatacaattaggcagtttagcgaaaaagacacttgccgatacaagtaacgataccaaaagaattggtctatcattagattgttccagaacatattattctccttctacaatcaaaaagtatatagatttattaaagaaagatcatggtacatatcttcaattacacttaaatgacaatgaaagatatggtgttgaaagttcaacgttaggacaaacaacgcaaaacgctacacttaaagatggtgtttattacaataataaaacacacttagcatttttaagtaaaaatcaattattagatgtaattcaatacggttacactcatggaattgaagtaattccagaaatagacttacctggacatgctcaatctatatttaagcttctttcatatacttcagaaggaaagaaactagttaaagagttagaaaataaagatggttacaatgaaatgtactacaacaaacaagctacgattgatttttcaaaaaagcttttaagtgaatatgttggcatgcttcccagtggataccacattattgtaggtgccgatgaaataactattagtgataaaagtgatcaagaagccgttgttaagtatattaatgccattgatgattatgttaatgctaatcatttaaaacttgaaatgtggaatgatagttttcataaggcggttttaagtaaatatcataaagatattttaattaattactggagtttaacaggtgaagttagctcaagtaaggatagaaaagacaacatcaggatgagagcaacacttcctgaattaaataaggctggttttaagacaattaactacaatagttattatctatatatgattacagatccaacatcatttaccaatgaatctaagaaaatttggacttccgagtttaaaaaatggaaaatgaatatgtggaatgatgaatctacaaaagatatcacaaagagcgccaataatattggtgctgccatatcaatatggggtgaatatccaaatcaatatactggtgatcaaacatataataagacatattattacgttgatacgtttttaaaggcccaggataaatttactaagtaa

SEQ ID NO: 5 - protein, 381 aa, Lactobacillus apinorum
MRNKRFIIVGMILFLVLMFIQLGSLAKKTLADTSNDTKRIGLSLDCSRTYYSPSTIKKYIDLLKKDHGTYLQLHLNDNERYGVESSTLGQTTQNATLKDGVYYNNKTHLAFLSKNQLLDVIQYGYTHGIEVIPEIDLPGHAQSIFKLLSYTSEGKKLVKELENKDGYNEMYYNKQATIDFSKKLLSEYVGMLPSGYHIIVGADEITISDKSDQEAVVKYINAIDDYVNANHLKLEMWNDSFHKAVLSKYHKDILINYWSLTGEVSSSKDRKDNIRMRATLPELNKAGFKTINYNSYYLYMITDPTSFTNESKKIWTSEFKKWKMNMWNDESTKDITKSANNIGAAISIWGEYPNQYTGDQTYNKTYYYVDTFLKAQDKFTK

SEQ ID NO: 6 - protein, 353 aa, Lactobacillus apinorum
TLADTSNDTKRIGLSLDCSRTYYSPSTIKKYIDLLKKDHGTYLQLHLNDNERYGVESSTLGQTTQNATLKDGVYYNNKTHLAFLSKNQLLDVIQYGYTHGIEVIPEIDLPGHAQSIFKLLSYTSEGKKLVKELENKDGYNEMYYNKQATIDFSKKLLSEYVGMLPSGYHIIVGADEITISDKSDQEAVVKYINAIDDYVNANHLKLEMWNDSFHKAVLSKYHKDILINYWSLTGEVSSSKDRKDNIRMRATLPELNKAGFKTINYNSYYLYMITDPTSFTNESKKIWTSEFKKWKMNMWNDESTKDITKSANNIGAAISIWGEYPNQYTGDQTYNKTYYYVDTFLKAQDKFTK

SEQ ID NO: 7 - DNA, 1086 bp, Lactobacillus paraplantarum
  CDS (1)..(1083)
  sig_peptide (1)..(90)
  mat_peptide (91)..(1083)
atgaagtgccgacattactttacacaactattaatatttattagcccgctgattcttctttgcttcagccagccccgtacggcaactgccaattcatcaacattgaatactagtcaaggggtcatgttagatttaggtcgccatccgttagatgaaactgcaattaaagccgtcattagtgctgctgccgaacaacacatgcaatacgtcgaactacacttatcagataacgaacatctatgctttcaatcggcttatttaggtaatgccgcatcggcaaccgtattatcggcaacgactttagaacagctagttgcttatgccaatcagttgaacattgaactagttcctgatgttgaccttccctcgcacgcgggagccattttacgccaattgcaacaaactcatcccgatatttacaataccgttaagttggatgacgaaaccatcgactatactaaaccggcagcagtcagtctcgctaccacactttatggcgagctcgatgctagttttaacaatcaaagccagcacgatttgatgctcggcgctgatgaggtttctggcagcgctagcgcctatatcgaactgaccacctttatcaatcaggtcagtcgatttcaaaatcaaaacggcttcaacactagtatttggaatgattcgctattaaaaaatgaactcaatcgtctggattcaaacattacaatcaattactggtcacaatctggtaacaataccgatgcggctatcattgccgaccgctatgccaaccgtgcatccgttcccgacattttagcctctgggcatccgatcgtgaactgtaatagttatgcgacctattatcaattcaaaaatattggcaatgtcaatgatgacaattactttattaattatcttaatcacacctttcgcccgaatatctttaacgaaattgacaccaacgggcataatcaggattggaccattgaagatggcgtcacaactaacggtatcttagttagcttgtggggggccgattcagagcatgttacaccaactgctattgtcaatttcattaaacgtatggcgattccccggtcattttaa

SEQ ID NO: 8 - protein, 361 aa, Lactobacillus paraplantarum
MKCRHYFTQLLIFISPLILLCFSQPRTATANSSTLNTSQGVMLDLGRHPLDETAIKAVISAAAEQHMQYVELHLSDNEHLCFQSAYLGNAASATVLSATTLEQLVAYANQLNIELVPDVDLPSHAGAILRQLQQTHPDIYNTVKLDDETIDYTKPAAVSLATTLYGELDASFNNQSQHDLMLGADEVSGSASAYIELTTFINQVSRFQNQNGFNTSIWNDSLLKNELNRLDSNITINYWSQSGNNTDAAIIADRYANRASVPDILASGHPIVNCNSYATYYQFKNIGNVNDDNYFINYLNHTFRPNIFNEIDTNGHNQDWTIEDGVTTNGILVSLWGADSEHVTPTAIVNFIKRMAIPRSF

SEQ ID NO: 9 - protein, 331 aa, Lactobacillus paraplantarum
NSSTLNTSQGVMLDLGRHPLDETAIKAVISAAAEQHMQYVELHLSDNEHLCFQSAYLGNAASATVLSATTLEQLVAYANQLNIELVPDVDLPSHAGAILRQLQQTHPDIYNTVKLDDETIDYTKPAAVSLATTLYGELDASFNNQSQHDLMLGADEVSGSASAYIELTTFINQVSRFQNQNGFNTSIWNDSLLKNELNRLDSNITINYWSQSGNNTDAAIIADRYANRASVPDILASGHPIVNCNSYATYYQFKNIGNVNDDNYFINYLNHTFRPNIFNEIDTNGHNQDWTIEDGVTTNGILVSLWGADSEHVTPTAIVNFIKRMAIPRSF

SEQ ID NO: 10 - protein, 27 aa, artificial
  Signal peptide
MKKPLGKIVASTALLISVAFSSSIASA

SEQ ID NO: 11 - protein, 8 aa, artificial
  His-tag
HHHHHHPR

SEQ ID NO: 12 - protein, 4 aa, artificial
  motif
  misc (2)..(2): Xaa= any natural occuring amino acids
GXDE

SEQ ID NO: 13 - protein, 7 aa, artificial
  motif
  misc (1)..(1): Xaa = E (Glu) or Q (Gln)
  misc (2)..(2): Xaa = N (Asn) or R (Arg) or S (Ser) or H (His) or A (Ala)
  misc (3)..(3): Xaa = Y (Tyr) or V (Val) or F (Phe) or L (Leu)
  misc (4)..(4): Xaa = A (Ala) or G (Gly) or S (Ser) or T (Thr) or C (Cys)
  misc (5)..(5): Xaa =I (Ile) or V (Val) or L (Leu) or F (Phe)
  misc (6)..(6): Xaa =E (Glu) or A (Ala) or Q (Gln) or Y (Tyr) or N (Asn)
  misc (7)..(7): Xaa =S(Ser) or N (Asn)
XXXXXXX

SEQ ID NO: 14 - protein, 8 aa, artificial
  motif
  misc (1)..(1): Xaa = V(Val) or L (Leu) or I (Ile) or M (Met)
  misc (2)..(2): Xaa = L (Leu) or I (Ile) or V(Val)
  misc (4)..(4): Xaa = G (Gly) or A (Ala) or V (Val)
  misc (7)..(7): Xaa = V (Val) or I (Ile)
  misc (8)..(8): Xaa = P (Pro) or S (Ser) or A (Ala)
XXGXDEXX

SEQ ID NO: 15 - protein, 7 aa, artificial
  SEQ ID NO 15
  misc (1)..(1): Xaa = G(Gly) or K (Lys)
  misc (3)..(3): Xaa = I (Ile) or L (Leu)
  misc (4)..(4): Xaa = I (Ile) or L (Leu)
  misc (5)..(5): Xaa = K (Lys) or S (Ser) or R (Arg)
  misc (6)..(6): Xaa = L(Leu) or Q(Gln)
XAXXXXL

SEQ ID NO: 16 - DNA, 1524 bp, Streptococcus merionis
  CDS (1)..(1521)
  sig_peptide (1)..(75)
  mat_peptide (76)..(1521)
atgcataaggttaaggtacttttagggacggttctgctctttttaacactattgttgacaggacagccagaggcacaagaacctatcgttaaactctcaggcggagtgatggtggatgtggctaggagatattactctctaaactctctgaaatctatcattgatactgtttcggagaataaaggagactttgttcatctccacttgacagatgatcaaaattatgggttggagagtcagtttctcaatcaaacagcttcaaatgcaatctataatcaagatgatcaaagctatactaatcctaatacgaatcgaaaatttctcagttatggacagttggctgagcttaaaagttatgcgggttcaaaaggcatccgattgataccagaaattgacaccccagctcatacaggagggctaaaggccttgcttccctacgctgagccagcagttactagtcaatttaagtgggtatcttgggacgaagataggcaactagatcttgatgcagctactactcaggaagctgttagacagttatatatggaactagtccgagaattgcctggcttagagtatatccatattggaggcgatgaaatttctggaggacttatacaaggccagtctttcattagtcatgtgaatcagttatgcgactatttagcaggtcaaggtatcaaaactcaaatatggaatgatagcttatcccgtcaactgctaccttctttaaatcgtaacgttgagattgcttattgggggtatcttcctcacagaaatccagatttagcaacagcttctgaccttagtgatcaggattttaagctccttaattataatgggtattatctagcttttgttcctaagccctcagaaaaacttcaatcggatgccctatttgcagcaaatgatattctaaagacttggaatctttcccagtttcatatggatacgggtgattccattaatagtttaaagaatgtcattggagcggctttttccatatggagtgaagagtcagctggtctgactgacgaggagatattttctgccatgggtagtccgattcgagctcttttgacagttatcaatcaagaaaatataaagagaaacgagaatacgacaactaccaccaccgagtcaatgactgaggctacgacaactattacaactgagccgacaacccaatcaaccacagaaagtacgacaactactacaaccgagtcaacgacagagactacgacaactgtcacaactgagtcaacaactaagtcgaccacagaaggcacgacagaaacaacaacccctatcccaccaatgcctcagcctacaacgtctcctgagacaagtacagctacacatgcaacaacgactaacccaagtacatcaaaagatggcaataaactgtctaaatcaaaacggatattgccaagtacaggtgaaacgattggtgtcctttcagtagcaggattggcgctcttcttgtttgttgggcttacatattaccgtcacaagaagaattaa

SEQ ID NO: 17 - protein, 507 aa, Streptococcus merionis
MHKVKVLLGTVLLFLTLLLTGQPEAQEPIVKLSGGVMVDVARRYYSLNSLKSIIDTVSENKGDFVHLHLTDDQNYGLESQFLNQTASNAIYNQDDQSYTNPNTNRKFLSYGQLAELKSYAGSKGIRLIPEIDTPAHTGGLKALLPYAEPAVTSQFKWVSWDEDRQLDLDAATTQEAVRQLYMELVRELPGLEYIHIGGDEISGGLIQGQSFISHVNQLCDYLAGQGIKTQIWNDSLSRQLLPSLNRNVEIAYWGYLPHRNPDLATASDLSDQDFKLLNYNGYYLAFVPKPSEKLQSDALFAANDILKTWNLSQFHMDTGDSINSLKNVIGAAFSIWSEESAGLTDEEIFSAMGSPIRALLTVINQENIKRNENTTTTTTESMTEATTTITTEPTTQSTTESTTTTTTESTTETTTTVTTESTTKSTTEGTTETTTPIPPMPQPTTSPETSTATHATTTNPSTSKDGNKLSKSKRILPSTGETIGVLSVAGLALFLFVGLTYYRHKKN

SEQ ID NO: 18 - protein, 482 aa, Streptococcus merionis
QEPIVKLSGGVMVDVARRYYSLNSLKSIIDTVSENKGDFVHLHLTDDQNYGLESQFLNQTASNAIYNQDDQSYTNPNTNRKFLSYGQLAELKSYAGSKGIRLIPEIDTPAHTGGLKALLPYAEPAVTSQFKWVSWDEDRQLDLDAATTQEAVRQLYMELVRELPGLEYIHIGGDEISGGLIQGQSFISHVNQLCDYLAGQGIKTQIWNDSLSRQLLPSLNRNVEIAYWGYLPHRNPDLATASDLSDQDFKLLNYNGYYLAFVPKPSEKLQSDALFAANDILKTWNLSQFHMDTGDSINSLKNVIGAAFSIWSEESAGLTDEEIFSAMGSPIRALLTVINQENIKRNENTTTTTTESMTEATTTITTEPTTQSTTESTTTTTTESTTETTTTVTTESTTKSTTEGTTETTTPIPPMPQPTTSPETSTATHATTTNPSTSKDGNKLSKSKRILPSTGETIGVLSVAGLALFLFVGLTYYRHKKN